European Patent Application EP 4 218 793 A2, published August 2, 2023. Title: Compound and compositions for multitarget treatment of tau protein-related disorders. Applicant: Fondazione IRCCS Istituto Neurologico Carlo Besta. The sequence listing filed with the application follows.

SEQUENCE LISTING (1 sequence)

SEQ ID NO: 1 - protein, 6 aa, unidentified
  REGION 1..6: note = A1beta-6A2V(D)
DVEFRH